European Patent Application EP 4 582 546 A1, published July 9, 2025. Title: ADENO-ASSOCIATED VIRUS STRUCTURAL PLASMID CAPABLE OF IMPROVING ADENO-ASSOCIATED VIRUS TITER. Applicant: Jiangsu GenScript Probio Biotech Co., Ltd. The sequence listing filed with the application follows.

SEQUENCE LISTING (10 sequences)

SEQ ID NO: 1 - DNA, 148 bp, synthetic construct
  source 1..148: mol_type = other DNA; note = P5 promoter
ggtggagtcgtgacgtgaattacgtcatagggttagggaggtcctgtattagaggtcacgtgagtgttttgcgacattttgcgacaccatgtggtcacgctgggtatttaagcccgagtgagcacgcagggtctccattttgaagcgg

SEQ ID NO: 2 - DNA, 180 bp, synthetic construct
  source 1..180: mol_type = other DNA; note = P40 promoter
ggtcaccaagcaggaagtcaaagactttttccggtgggcaaaggatcacgtggttgaggtggagcatgaattctacgtcaaaaagggtggagccaagaaaagacccgcccccagtgacgcagatataagtgagcccaaacgggtgcgcgagtcagttgcgcagccatcgacgtcagacgc

SEQ ID NO: 3 - DNA, 508 bp, synthetic construct
  source 1..508: mol_type = other DNA; note = CMV promoter
cgttacataacttacggtaaatggcccgcctggctgaccgcccaacgacccccgcccattgacgtcaataatgacgtatgttcccatagtaacgccaatagggactttccattgacgtcaatgggtggagtatttacggtaaactgcccacttggcagtacatcaagtgtatcatatgccaagtacgccccctattgacgtcaatgacggtaaatggcccgcctggcattatgcccagtacatgaccttatgggactttcctacttggcagtacatctacgtattagtcatcgctattaccatgctgatgcggttttggcagtacatcaatgggcgtggatagcggtttgactcacggggatttccaagtctccaccccattgacgtcaatgggagtttgttttggcaccaaaatcaacgggactttccaaaatgtcgtaacaactccgccccattgacgcaaatgggcggtaggcgtgtacggtgggaggtctatataagcagagct

SEQ ID NO: 4 - DNA, 82 bp, synthetic construct
  source 1..82: mol_type = other DNA; note = SV40 poly(A)
aacttgtttattgcagcttataatggttacaaataaagcaatagcatcacaaatttcacaaataaagcatttttttcactgc

SEQ ID NO: 5 - DNA, 208 bp, synthetic construct
  source 1..208: mol_type = other DNA; note = BGH poly(A)
ctgtgccttctagttgccagccatctgttgtttgcccctcccccgtgccttccttgaccctggaaggtgccactcccactgtcctttcctaataaaatgaggaaattgcatcgcattgtctgagtaggtgtcattctattctggggggtggggtggggcaggacagcaagggggaggattgggaagacaatagcaggcatgctgggga

SEQ ID NO: 6 - DNA, 150 bp, synthetic construct
  source 1..150: mol_type = other DNA; note = P19 promoter
gccggaggcgggaacaaggtggtggatgagtgctacatccccaattacttgctccccaaaacccagcctgagctccagtgggcgtggactaatatggaacagtatttaagcgcctgtttgaatctcacggagcgtaaacggttggtggcg

SEQ ID NO: 7 - DNA, 180 bp, synthetic construct
  source 1..180: mol_type = other DNA; note = DelP40 promoter
ggtcaccaagcaagaggttaaggactttttccggtgggcaaaggatcacgtggttgaggtggagcatgaattctacgtcaaaaagggtggagccaagaaaagaccagcaccaagtgacgcagacatcagcgagcccaaacgggtgcgcgagtcagttgcgcagccatcgacgtcagacgc

SEQ ID NO: 8 - DNA, 793 bp, synthetic construct
  source 1..793: mol_type = other DNA; note = CBh promoter
cgttacataacttacggtaaatggcccgcctggctgaccgcccaacgacccccgcccattgacgtcaatagtaacgccaatagggactttccattgacgtcaatgggtggagtatttacggtaaactgcccacttggcagtacatcaagtgtatcatatgccaagtacgccccctattgacgtcaatgacggtaaatggcccgcctggcattgtgcccagtacatgaccttatgggactttcctacttggcagtacatctacgtattagtcatcgctattaccatggtcgaggtgagccccacgttctgcttcactctccccatctcccccccctccccacccccaattttgtatttatttattttttaattattttgtgcagcgatgggggcggggggggggggggggcgcgcgccaggcggggcggggcggggcgaggggcggggcggggcgaggcggagaggtgcggcggcagccaatcagagcggcgcgctccgaaagtttccttttatggcgaggcggcggcggcggcggccctataaaaagcgaagcgcgcggcgggcgggagtcgctgcgcgctgccttcgccccgtgccccgctccgccgccgcctcgcgccgcccgccccggctctgactgaccgcgttactcccacaggtgagcgggcgggacggcccttctcctccgggctgtaattagctgagcaagaggtaagggtttaagggatggttggttggtggggtattaatgtttaattacctggagcacctgcctgaaatcactttttttcag

SEQ ID NO: 9 - DNA, 1602 bp, synthetic construct
  source 1..1602: mol_type = other DNA; note = CAG promoter
cgttacataacttacggtaaatggcccgcctggctgaccgcccaacgacccccgcccattgacgtcaataatgacgtatgttcccatagtaacgccaatagggactttccattgacgtcaatgggtggagtatttacggtaaactgcccacttggcagtacatcaagtgtatcatatgccaagtacgccccctattgacgtcaatgacggtaaatggcccgcctggcattatgcccagtacatgaccttatgggactttcctacttggcagtacatctacgtattagtcatcgctattaccatgatggtcgaggtgagccccacgttctgcttcactctccccatctcccccccctccccacccccaattttgtatttatttattttttaattattttgtgcagcgatgggggcggggggggggggggggcgcgcgcaggcggggcggggcggggcgaggggcggggcggggcgaggcggagaggtgcggcggcagccaatcagagcggcgcgctccgaaagtttccttttatggcgaggcggcggcggcggcggccctataaaaagcgaagcgcgcggcgggcgggagtcgctgcgcgctgccttcgccccgtgccccgctccgccgccgcctcgcgccgcccgccccggctctgactgaccgcgttactcccacaggtgagcgggcgggacggcccttctcctccgggctgtaattagcgcttggtttaatgacggcttgtttcttttctgtggctgcgtgaaagccttgaggggctccgggagggccctttgtgcggggggagcggctcggggggtgcgtgcgtgtgtgtgtgcgtggggagcgccgcgtgcggctccgcgctgcccggcggctgtgagcgctgcgggcgcggcgcggggctttgtgcgctccgcagtgtgcgcgaggggagcgcggccgggggcggtgccccgcggtgcggggggggctgcgaggggaacaaaggctgcgtgcggggtgtgtgcgtgggggggtgagcagggggtgtgggcgcgtcggtcgggctgcaaccccccctgcacccccctccccgagttgctgagcacggcccggcttcgggtgcggggctccgtacggggcgtggcgcggggctcgccgtgccgggcggggggtggcggcaggtgggggtgccgggcggggcggggccgcctcgggccggggagggctcgggggaggggcgcggcggcccccggagcgccggcggctgtcgaggcgcggcgagccgcagccattgccttttatggtaatcgtgcgagagggcgcagggacttcctttgtcccaaatctgtgcggagccgaaatctgggaggcgccgccgcaccccctctagcgggcgcggggcgaagcggtgcggcgccggcaggaaggaaatgggcggggagggccttcgtgcgtcgccgcgccgccgtccccttctccctctccagcctcggggctgtccgcggggggacggctgccttcgggggggacggggcagggcggggttcggcttctggcgtgtgaccggcggctctagagcctctgctaaccatgttcatgccttcttctttttcctacag

SEQ ID NO: 10 - DNA, 212 bp, synthetic construct
  source 1..212: mol_type = other DNA; note = EF1alpha promoter
gggcagagcgcacatcgcccacagtccccgagaagttggggggaggggtcggcaattgaaccggtgcctagagaaggtggcgcggggtaaactgggaaagtgatgtcgtgtactggctccgcctttttcccgagggtgggggagaaccgtatataagtgcagtagtcgccgtgaacgttctttttcgcaacgggtttgccgccagaacacag